European Patent Application EP 4 349 371 A1, published April 10, 2024. Title: DRUG CONJUGATE AND USE THEREOF. Applicant: Bio-Thera Solutions, Ltd. Application PCT/CN/2022/096690. The sequence listing filed with the application follows.

SEQUENCE LISTING (26 sequences)

SEQ ID NO: 1 - protein, 447 aa, Artificial Sequence
  heavy chain of the anti-EGFR antibody
QVQESGPGLVKPSETLSLTCTVSGGSVSSGDYYWTWIRQSPGKGLEWIGHIYYSGNTNYNPSLKSRLTISIDTSKTQFSLKLSSVTAADTAIYYCVRDRVTGAFDIWGQGTLVTVSSASTKGPSVFPLAPSSKSTSGGTAALGCLVKDYFPEPVTVSWNSGALTSGVHTFPAVLQSSGLYSLSSVVTVPSSSLGTQTYICNVNHKPSNTKVDKKVEPKSCDKTHTCPPCPAPELLGGPSVFLFPPKPKDTLMISRTPEVTCVVVDVSHEDPEVKFNWYVDGVEVHNAKTKPREEQYNSTYRVVSVLTVLHQDWLNGKEYKCKVSNKALPAPIEKTISKAKGQPREPQVYTLPPSRDELTKNQVSLTCLVKGFYPSDIAVEWESNGQPENNYKTTPPVLDSDGSFFLYSKLTVDKSRWQQGNVFSCSVMHEALHNHYTQKSLSLSPGK

SEQ ID NO: 2 - protein, 214 aa, Artificial Sequence
  light chain of the anti-EGFR antibody
DIQMTQSPSSLSASVGDRVTITCQASQDISNYLNWYQQKPGKAPKLLIYDASNLETGVPSRFSGSGSGTDFTFTISSLQPEDIATYFCQHFDHLPLAFGGGTKVEIKRTVAAPSVFIFPPSDEQLKSGTASVVCLLNNFYPREAKVQWKVDNALQSGNSQESVTEQDSKDSTYSLSSTLTLSKADYEKHKVYACEVTHQGLSSPVTKSFNRGEC

SEQ ID NO: 3 - protein, 450 aa, Artificial Sequence
  heavy chain of the anti-HER2 antibody
EVQLVESGGGLVQPGGSLRLSCAASGFNIKDTYIHWVRQAPGKGLEWVARIYPTNGYTRYADSVKGRFTISADTSKNTAYLQMNSLRAEDTAVYYCSRWGGDGFYAMDYWGQGTLVTVSSASTKGPSVFPLAPSSKSTSGGTAALGCLVKDYFPEPVTVSWNSGALTSGVHTFPAVLQSSGLYSLSSVVTVPSSSLGTQTYICNVNHKPSNTKVDKKVEPKSCDKTHTCPPCPAPELLGGPSVFLFPPKPKDTLMISRTPEVTCVVVDVSHEDPEVKFNWYVDGVEVHNAKTKPREEQYNSTYRVVSVLTVLHQDWLNGKEYKCKVSNKALPAPIEKTISKAKGQPREPQVYTLPPSREEMTKNQVSLTCLVKGFYPSDIAVEWESNGQPENNYKTTPPVLDSDGSFFLYSKLTVDKSRWQQGNVFSCSVMHEALHNHYTQKSLSLSPGK

SEQ ID NO: 4 - protein, 214 aa, Artificial Sequence
  light chain of the anti-HER2 antibody
DIQMTQSPSSLSASVGDRVTITCRASQDVNTAVAWYQQKPGKAPKLLIYSASFLYSGVPSRFSGSRSGTDFTLTISSLQPEDFATYYCQQHYTTPPTFGQGTKVEIKRTVAAPSVFIFPPSDEQLKSGTASVVCLLNNFYPREAKVQWKVDNALQSGNSQESVTEQDSKDSTYSLSSTLTLSKADYEKHKVYACEVTHQGLSSPVTKSFNRGEC

SEQ ID NO: 5 - protein, 451 aa, Artificial Sequence
  heavy chain of the hRS9 antibody
QVQLQQSGSELKKPGASVKVSCKASGYTFTNYGMNWVKQAPGQGLKWMGWINTYTGEPTYTDDFKGRFAFSLDTSVSTAYLQISSLKADDTAVYFCARGGFGSSYWYFDVWGQGTLVTVSSASTKGPSVFPLAPSSKSTSGGTAALGCLVKDYFPEPVTVSWNSGALTSGVHTFPAVLQSSGLYSLSSVVTVPSSSLGTQTYICNVNHKPSNTKVDKKVEPKSCDKTHTCPPCPAPELLGGPSVFLFPPKPKDTLMISRTPEVTCVVVDVSHEDPEVKFNWYVDGVEVHNAKTKPREEQYNSTYRVVSVLTVLHQDWLNGKEYKCKVSNKALPAPIEKTISKAKGQPREPQVYTLPPSRDELTKNQVSLTCLVKGFYPSDIAVEWESNGQPENNYKTTPPVLDSDGSFFLYSKLTVDKSRWQQGNVFSCSVMHEALHNHYTQKSLSLSPGK

SEQ ID NO: 6 - protein, 214 aa, Artificial Sequence
  light chain of the hRS9 antibody
DIQLTQSPSSLSASVGDRVSITCKASQDVSIAVAWYQQKPGKAPKLLIYSASYRYTGVPDRFSGSGSGTDFTLTISSLQPEDFAVYYCQQHYITPLTFGAGTKVEIKRTVAAPSVFIFPPSDEQLKSGTASVVCLLNNFYPREAKVQWKVDNALQSGNSQESVTEQDSKDSTYSLSSTLTLSKADYEKHKVYACEVTHQGLSSPVTKSFNRGEC

SEQ ID NO: 7 - protein, 5 aa, Artificial Sequence
  VH CDR1 of the anti-CLND18.2 antibody
DYGMH

SEQ ID NO: 8 - protein, 17 aa, Artificial Sequence
  VH CDR2 of the anti-CLND18.2 antibody
YISRGRSTTYSTDTVKG

SEQ ID NO: 9 - protein, 10 aa, Artificial Sequence
  VH CDR3 of the anti-CLND18.2 antibody
GSYYGNALDY

SEQ ID NO: 10 - protein, 17 aa, Artificial Sequence
  VL CDR1 of the anti-CLND18.2 antibody
KSSQSLLNSGNQRNYLT

SEQ ID NO: 11 - protein, 7 aa, Artificial Sequence
  VL CDR2 of the anti-CLND18.2 antibody
WASTRES

SEQ ID NO: 12 - protein, 9 aa, Artificial Sequence
  VL CDR3 of the anti-CLND18.2 antibody
QSAYSYPFT

SEQ ID NO: 13 - protein, 119 aa, Artificial Sequence
  heavy chain variable region of the anti-CLND18.2 antibody
EVQLLESGGGLVQPGGSLRLSCAASGFTFSDYGMHWVRQAPGKGLEWVAYISRGRSTTYSTDTVKGRFTISRDNSKNTLYLQMNSLRAEDTAVYYCARGSYYGNALDYWGQGTLVTVSS

SEQ ID NO: 14 - protein, 113 aa, Artificial Sequence
  light chain variable region of the anti-CLND18.2 antibody
DIVMTQSPDSLAVSLGERATINCKSSQSLLNSGNQRNYLTWYQQKPGQPPKLLIYWASTRESGVPDRFSGSGSGTDFTLTISSLQAEDVAVYYCQSAYSYPFTFGGGTKLEIK

SEQ ID NO: 15 - protein, 330 aa, Artificial Sequence [sequence omitted]

SEQ ID NO: 16 - protein, 330 aa, Artificial Sequence
  heavy chain constant region of the anti-CLND18.2 antibody
ASTKGPSVFPLAPSSKSTSGGTAALGCLVKDYFPEPVTVSWNSGALTSGVHTFPAVLQSSGLYSLSSVVTVPSSSLGTQTYICNVNHKPSNTKVDKKVEPKSCDKTHTCPPCPAPELLGGPSVFLFPPKPKDTLMISRTPEVTCVVVDVSHEDPEVKFNWYVDGVEVHNAKTKPREEQYASTYRVVSVLTVLHQDWLNGKEYKCKVSNKALPAPIEKTISKAKGQPREPQVYTLPPSRDELTKNQVSLTCLVKGFYPSDIAVEWESNGQPENNYKTTPPVLDSDGSFFLYSKLTVDKSRWQQGNVFSCSVMHEALHNHYTQKSLSLSPGK

SEQ ID NO: 17 - protein, 107 aa, Artificial Sequence [sequence omitted]

SEQ ID NO: 18 - protein, 449 aa, Artificial Sequence
  heavy chain of the anti-CLND18.2 antibody
EVQLLESGGGLVQPGGSLRLSCAASGFTFSDYGMHWVRQAPGKGLEWVAYISRGRSTTYSTDTVKGRFTISRDNSKNTLYLQMNSLRAEDTAVYYCARGSYYGNALDYWGQGTLVTVSSASTKGPSVFPLAPSSKSTSGGTAALGCLVKDYFPEPVTVSWNSGALTSGVHTFPAVLQSSGLYSLSSVVTVPSSSLGTQTYICNVNHKPSNTKVDKKVEPKSCDKTHTCPPCPAPELLGGPSVFLFPPKPKDTLMISRTPEVTCVVVDVSHEDPEVKFNWYVDGVEVHNAKTKPREEQYNSTYRVVSVLTVLHQDWLNGKEYKCKVSNKALPAPIEKTISKAKGQPREPQVYTLPPSRDELTKNQVSLTCLVKGFYPSDIAVEWESNGQPENNYKTTPPVLDSDGSFFLYSKLTVDKSRWQQGNVFSCSVMHEALHNHYTQKSLSLSPGK

SEQ ID NO: 19 - protein, 449 aa, Artificial Sequence
  heavy chain of the anti-CLND18.2 antibody
EVQLLESGGGLVQPGGSLRLSCAASGFTFSDYGMHWVRQAPGKGLEWVAYISRGRSTTYSTDTVKGRFTISRDNSKNTLYLQMNSLRAEDTAVYYCARGSYYGNALDYWGQGTLVTVSSASTKGPSVFPLAPSSKSTSGGTAALGCLVKDYFPEPVTVSWNSGALTSGVHTFPAVLQSSGLYSLSSVVTVPSSSLGTQTYICNVNHKPSNTKVDKKVEPKSCDKTHTCPPCPAPELLGGPSVFLFPPKPKDTLMISRTPEVTCVVVDVSHEDPEVKFNWYVDGVEVHNAKTKPREEQYASTYRVVSVLTVLHQDWLNGKEYKCKVSNKALPAPIEKTISKAKGQPREPQVYTLPPSRDELTKNQVSLTCLVKGFYPSDIAVEWESNGQPENNYKTTPPVLDSDGSFFLYSKLTVDKSRWQQGNVFSCSVMHEALHNHYTQKSLSLSPGK

SEQ ID NO: 20 - protein, 220 aa, Artificial Sequence
  light chain of the anti-CLND18.2 antibody
DIVMTQSPDSLAVSLGERATINCKSSQSLLNSGNQRNYLTWYQQKPGQPPKLLIYWASTRESGVPDRFSGSGSGTDFTLTISSLQAEDVAVYYCQSAYSYPFTFGGGTKLEIKRTVAAPSVFIFPPSDEQLKSGTASVVCLLNNFYPREAKVQWKVDNALQSGNSQESVTEQDSKDSTYSLSSTLTLSKADYEKHKVYACEVTHQGLSSPVTKSFNRGEC

SEQ ID NO: 21 - protein, 445 aa, Artificial Sequence
  heavy chain of the anti-B7H3 antibody A
EVQLVQSGAEVKKSGESLKISCKASGYTFTDYDINWVRQMPGKGLEWIGWIFPGDDTTKYNEKFKGQVTLSADKSTNTAYMQWSSLKASDTAMYYCARSPSFDYWGQGTLVTVSSASTKGPSVFPLAPSSKSTSGGTAALGCLVKDYFPEPVTVSWNSGALTSGVHTFPAVLQSSGLYSLSSVVTVPSSSLGTQTYICNVNHKPSNTKVDKKVEPKSCDKTHTCPPCPAPELLGGPSVFLFPPKPKDTLMISRTPEVTCVVVDVSHEDPEVKFNWYVDGVEVHNAKTKPREEQYNSTYRVVSVLTVLHQDWLNGKEYKCKVSNKALPAPIEKTISKAKGQPREPQVYTLPPSRDELTKNQVSLTCLVKGFYPSDIAVEWESNGQPENNYKTTPPVLDSDGSFFLYSKLTVDKSRWQQGNVFSCSVMHEALHNHYTQKSLSLSPGK

SEQ ID NO: 22 - protein, 212 aa, Artificial Sequence
  light chain of the anti-B7H3 antibody A
QIVLTQSPGTLSLSPGERATLSCSASSTIGFMYWYQQKPGQAPRRWIYDTSKLASGVPDRFSGSGSGTDYTLTISRLEPEDFAVYYCHQRSSYPTFGQGTKVEIKRTVAAPSVFIFPPSDEQLKSGTASVVCLLNNFYPREAKVQWKVDNALQSGNSQESVTEQDSKDSTYSLSSTLTLSKADYEKHKVYACEVTHQGLSSPVTKSFNRGEC

SEQ ID NO: 23 - protein, 448 aa, Artificial Sequence
  heavy chain of the anti-FR antibody A
QVQLVQSGVEVKKPGASVKVSCKASGYSFTGYFMNWVRQAPGQGLEWIGRIHPYDGDTFYNQNFKDKATLTVDKSTTTAYMELKSLQFDDTAVYYCTRYDGSRAMDYWGQGTTVTVSSASTKGPSVFPLAPSSKSTSGGTAALGCLVKDYFPEPVTVSWNSGALTSGVHTFPAVLQSSGLYSLSSVVTVPSSSLGTQTYICNVNHKPSNTKVDKKVEPKSCDKTHTCPPCPAPELLGGPSVFLFPPKPKDTLMISRTPEVTCVVVDVSHEDPEVKFNWYVDGVEVHNAKTKPREEQYNSTYRVVSVLTVLHQDWLNGKEYKCKVSNKALPAPIEKTISKAKGQPREPQVYTLPPSRDELTKNQVSLTCLVKGFYPSDIAVEWESNGQPENNYKTTPPVLDSDGSFFLYSKLTVDKSRWQQGNVFSCSVMHEALHNHYTQKSLSLSPGK

SEQ ID NO: 24 - protein, 218 aa, Artificial Sequence
  light chain of the anti-FR antibody A
EIVLTQSPATLSLSPGERATLSCKASQSVSFAGTSLMHWYQQKPGQAPRLLIYRASNLEAGVPARFSGSGSKTDFTLTISSLEPEDFAVYYCQQSREYPYTFGGGTKVEIKRTVAAPSVFIFPPSDEQLKSGTASVVCLLNNFYPREAKVQWKVDNALQSGNSQESVTEQDSKDSTYSLSSTLTLSKADYEKHKVYACEVTHQGLSSPVTKSFNRGEC

SEQ ID NO: 25 - protein, 261 aa, Artificial Sequence
  The full-length amino acid sequence of human CLDN18.2
MAVTACQGLGFVVSLIGIAGIIAATCMDQWSTQDLYNNPVTAVFNYQGLWRSCVRESSGFTECRGYFTLLGLPAMLQAVRALMIVGIVLGAIGLLVSIFALKCIRIGSMEDSAKANMTLTSGIMFIVSGLCAIAGVSVFANMLVTNFWMSTANMYTGMGGMVQTVQTRYTFGAALFVGWVAGGLTLIGGVMMCIACRGLAPEETNYKAVSYHASGHSVAYKPGGFKASTGFGSNTKNKKIYDGGARTEDEVQSYPSKHDYV

SEQ ID NO: 26 - DNA, 783 bp, Artificial Sequence
  The nucleic acid sequence of human CLDN18.2
atggccgtgactgcctgtcagggcttggggttcgtggtttcactgattgggattgcgggcatcattgctgccacctgcatggaccagtggagcacccaagacttgtacaacaaccccgtaacagctgttttcaactaccaggggctgtggcgctcctgtgtccgagagagctctggcttcaccgagtgccggggctacttcaccctgctggggctgccagccatgctgcaggcagtgcgagccctgatgatcgtaggcatcgtcctgggtgccattggcctcctggtatccatctttgccctgaaatgcatccgcattggcagcatggaggactctgccaaagccaacatgacactgacctccgggatcatgttcattgtctcaggtctttgtgcaattgctggagtgtctgtgtttgccaacatgctggtgactaacttctggatgtccacagctaacatgtacaccggcatgggtgggatggtgcagactgttcagaccaggtacacatttggtgcggctctgttcgtgggctgggtcgctggaggcctcacactaattgggggtgtgatgatgtgcatcgcctgccggggcctggcaccagaagaaaccaactacaaagccgtttcttatcatgcctcaggccacagtgttgcctacaagcctggaggcttcaaggccagcactggctttgggtccaacaccaaaaacaagaagatatacgatggaggtgcccgcacagaggacgaggtacaatcttatccttccaagcacgactatgtg